European Patent Specification EP 3 114 214 B1, published November 1, 2023. Title: IMPROVED REPROGRAMMING METHODS AND CELL CULTURE PLATFORMS. Applicant: VALAMEHR, Bahram FLYNN, Peter ABUJAROUR, Ramzey ROBINSON, Megan. The sequence listing filed with the application follows.

SEQUENCE LISTING (31 sequences)

SEQ ID NO: 1 - protein, 19 aa, Artificial Sequence
  Synthetic made in lab
LLNFDLLKLAGDVESNPGP

SEQ ID NO: 2 - protein, 19 aa, Artificial Sequence
  Synthetic made in lab
TLNFDLLKLAGDVESNPGP

SEQ ID NO: 3 - protein, 14 aa, Artificial Sequence
  Synthetic made in lab
LLKLAGDVESNPGP

SEQ ID NO: 4 - protein, 17 aa, Artificial Sequence
  Synthetic made in lab
NFDLLKLAGDVESNPGP

SEQ ID NO: 5 - protein, 20 aa, Artificial Sequence
  Synthetic made in lab
QLLNFDLLKLAGDVESNPGP

SEQ ID NO: 6 - protein, 24 aa, Artificial Sequence
  Synthetic made in lab
APVKQTLNFDLLKLAGDVESNPGP

SEQ ID NO: 7 - protein, 40 aa, Artificial Sequence
  Synthetic made in lab
VTELLYRMKRAETYCPRPLLAIHPTEARHKQKIVAPVKQT

SEQ ID NO: 8 - protein, 18 aa, Artificial Sequence
  Synthetic made in lab
LNFDLLKLAGDVESNPGP

SEQ ID NO: 9 - protein, 40 aa, Artificial Sequence
  Synthetic made in lab
LLAIHPTEARHKQKIVAPVKQTLNFDLLKLAGDVESNPGP

SEQ ID NO: 10 - protein, 33 aa, Artificial Sequence
  Synthetic made in lab
EARHKQKIVAPVKQTLNFDLLKLAGDVESNPGP

SEQ ID NO: 11 - DNA, 18 bp, Artificial Sequence
  Primer
gcccccaccctttgtgtt

SEQ ID NO: 12 - DNA, 23 bp, Artificial Sequence
  Primer
ttgaaaactttggcttccttgtt

SEQ ID NO: 13 - DNA, 20 bp, Artificial Sequence
  Primer
caggcccgaaagagaaagcg

SEQ ID NO: 14 - DNA, 20 bp, Artificial Sequence
  Primer
ggagggccttggaagcttag

SEQ ID NO: 15 - DNA, 20 bp, Artificial Sequence
  Primer
tatacacaggccgatgtggg

SEQ ID NO: 16 - DNA, 20 bp, Artificial Sequence
  Primer
ttgaccgggaccttgtcttc

SEQ ID NO: 17 - DNA, 20 bp, Artificial Sequence
  Primer
gtggtccgagtgtggttctg

SEQ ID NO: 18 - DNA, 20 bp, Artificial Sequence
  Primer
gttctcctgggccatcttgc

SEQ ID NO: 19 - DNA, 20 bp, Artificial Sequence
  Primer
aagcgcagatcaaaaggaga

SEQ ID NO: 20 - DNA, 20 bp, Artificial Sequence
  Primer
ccccctgaacctgaaacata

SEQ ID NO: 21 - DNA, 19 bp, Artificial Sequence
  Primer
tgcttcccgtatggctttc

SEQ ID NO: 22 - DNA, 22 bp, Artificial Sequence
  Primer
aaagggagatccgactcgtctg

SEQ ID NO: 23 - DNA, 20 bp, Artificial Sequence
  Primer
atcgtcaaagctgcacacag

SEQ ID NO: 24 - DNA, 20 bp, Artificial Sequence
  Primer
cccaggagtcccagtagtca

SEQ ID NO: 25 - DNA, 20 bp, Artificial Sequence
  Primer
gtggacctgacctgccgtct

SEQ ID NO: 26 - DNA, 20 bp, Artificial Sequence
  Primer
ggaggagtgggtgtcgctgt

SEQ ID NO: 27 - DNA, 24 bp, Artificial Sequenceq
  Primer
gggtttttgggattaagttcttca

SEQ ID NO: 28 - DNA, 22 bp, Artificial Sequence
  Primer
agcctaaatgatggtgcttggt

SEQ ID NO: 29 - protein, 7 aa, Artificial Sequence
  Polypeptide cleavage recognition site
  MISC_FEATURE (2)..(2): Xaa  represent any amino acid
  MISC_FEATURE (3)..(3): Xaa  represent any amino acid
  MISC_FEATURE (5)..(5): Xaa  represent any amino acid
  MISC_FEATURE (7)..(7): Xaa = Gly or Ser
EXXYXQX

SEQ ID NO: 30 - protein, 7 aa, Artificial Sequence
  Polypeptide cleavage recognition site
ENLYFQG

SEQ ID NO: 31 - protein, 7 aa, Artificial Sequence
  Polypeptide cleavage recognition site
ENLYFQS